European Patent Application EP 4 393 509 A1, published July 3, 2024. Title: ROS production enhancing agent. Applicant: Perseus Proteomics Inc. The sequence listing filed with the application follows.

SEQUENCE LISTING (42 sequences)

SEQ ID NO: 1 - protein, 5 aa, human
SYGMH

SEQ ID NO: 2 - protein, 17 aa, human
VISYDGSNKYYADSVKG

SEQ ID NO: 3 - protein, 14 aa, human
DSNFWSGYYSPVDV

SEQ ID NO: 4 - protein, 13 aa, human
TRSSGSIASNSVQ

SEQ ID NO: 5 - protein, 8 aa, human
YEDTQRPS

SEQ ID NO: 6 - protein, 10 aa, human
QSYDSAYHWV

SEQ ID NO: 7 - protein, 123 aa, human
DVQLVQSGGGVVQPGRSLRLSCAASGFPFKSYGMHWVRQAPGKGLEWVAVISYDGSNKYYADSVKGRFTISRDNSKNTLYLQMNSLRGEDTAVYYCARDSNFWSGYYSPVDVWGQGTTVTVSS

SEQ ID NO: 8 - protein, 111 aa, human
NFMLTQPHSVSESPGKTVTISCTRSSGSIASNSVQWYQQRPGSAPITVIYEDTQRPSGVPDRFSGSIDSSSNSASLTISGLQTEDEADYYCQSYDSAYHWVFGGGTKLAVL

SEQ ID NO: 9 - protein, 760 aa, human
MMDQARSAFSNLFGGEPLSYTRFSLARQVDGDNSHVEMKLAVDEEENADNNTKANVTKPKRCSGSICYGTIAVIVFFLIGFMIGYLGYCKGVEPKTECERLAGTESPVREEPGEDFPAARRLYWDDLKRKLSEKLDSTDFTGTIKLLNENSYVPREAGSQKDENLALYVENQFREFKLSKVWRDQHFVKIQVKDSAQNSVIIVDKNGRLVYLVENPGGYVAYSKAATVTGKLVHANFGTKKDFEDLYTPVNGSIVIVRAGKITFAEKVANAESLNAIGVLIYMDQTKFPIVNAELSFFGHAHLGTGDPYTPGFPSFNHTQFPPSRSSGLPNIPVQTISRAAAEKLFGNMEGDCPSDWKTDSTCRMVTSESKNVKLTVSNVLKEIKILNIFGVIKGFVEPDHYVVVGAQRDAWGPGAAKSGVGTALLLKLAQMFSDMVLKDGFQPSRSIIFASWSAGDFGSVGATEWLEGYLSSLHLKAFTYINLDKAVLGTSNFKVSASPLLYTLIEKTMQNVKHPVTGQFLYQDSNWASKVEKLTLDNAAFPFLAYSGIPAVSFCFCEDTDYPYLGTTMDTYKELIERIPELNKVARAAAEVAGQFVIKLTHDVELNLDYERYNSQLLSFVRDLNQYRADIKEMGLSLQWLYSARGDFFRATSRLTTDFGNAEKTDRFVMKKLNDRVMRVEYHFLSPYVSPKESPFRHVFWGSGSHTLPALLENLKLRKQNNGAFNETLFRNQLALATWTIQGAANALSGDVWDIDNEF

SEQ ID NO: 10 - protein, 28 aa, synthetic construct
  REGION 1..28: note = Description of Artificial Sequence: Recombinant tag
AAARGGPEQKLISEEDLNSAVDHHHHHH

SEQ ID NO: 11 - protein, 5 aa, human
SYWLS

SEQ ID NO: 12 - protein, 17 aa, human
KIDPSDSYTQYSPSFEG

SEQ ID NO: 13 - protein, 8 aa, human
HGYDAFHV

SEQ ID NO: 14 - protein, 13 aa, human
SGSSSNIGNNAVN

SEQ ID NO: 15 - protein, 7 aa, human
YDDLLPS

SEQ ID NO: 16 - protein, 11 aa, human
AAWDDSLNGWV

SEQ ID NO: 17 - protein, 5 aa, human
ELSMH

SEQ ID NO: 18 - protein, 17 aa, human
GFDPEDGETIYAQKFQG

SEQ ID NO: 19 - protein, 15 aa, human
DAYYGSGSPRDAFDI

SEQ ID NO: 20 - protein, 11 aa, human
GGDNVGGKSLH

SEQ ID NO: 21 - protein, 7 aa, human
DDRDRPS

SEQ ID NO: 22 - protein, 11 aa, human
QVWDDISRLVI

SEQ ID NO: 23 - protein, 5 aa, human
DYAMY

SEQ ID NO: 24 - protein, 17 aa, human
GINWNSAIIGYADSVKG

SEQ ID NO: 25 - protein, 11 aa, human
EALYYSAFFDS

SEQ ID NO: 26 - protein, 13 aa, human
SGSSSNIGNNYVS

SEQ ID NO: 27 - protein, 7 aa, human
DNNKRPS

SEQ ID NO: 28 - protein, 11 aa, human
GTWDSSLSAWV

SEQ ID NO: 29 - protein, 5 aa, human
DYAMH

SEQ ID NO: 30 - protein, 17 aa, human
GINWNGGSTDYADSVEG

SEQ ID NO: 31 - protein, 11 aa, human
DYADLGSGSDY

SEQ ID NO: 32 - protein, 13 aa, human
SGSRSNIGSNYVH

SEQ ID NO: 33 - protein, 7 aa, human
RNDQRPS

SEQ ID NO: 34 - protein, 11 aa, human
ASWDDKMSGRL

SEQ ID NO: 35 - protein, 117 aa, human
EVQLVESGAEVKKPGESLKISCKGSGYTFTSYWLSWVRQLPGKGLEWMGKIDPSDSYTQYSPSFEGQVTISADKSSNTAYLQWSSLKASDTAIYYCARHGYDAFHVWGQGTTVTVSR

SEQ ID NO: 36 - protein, 215 aa, human
QSVLTQPPSVSEAPRQRVTISCSGSSSNIGNNAVNWYQQLPGKAPKLLISYDDLLPSGVSDRFSGSTSGTSASLAISGLQSEDEADYYCAAWDDSLNGWVFGGGTKLTVLGQPKAAPSVTLFPPSSEELQANKATLVCLISDFYPGAVTVAWKADGSPVKAGVETTKPSKQSNNKYAASSYLSLTPEQWKSHRSYSCQVTHEGSTVEKTVAPTEC

SEQ ID NO: 37 - protein, 124 aa, human
QVQLQQSGAEVKKPGASVKVSCKVSGYTLTELSMHWVRQAPGKGLEWMGGFDPEDGETIYAQKFQGRVTMTEDTSTDTAYMELSSLRSEDTAVYYCATDAYYGSGSPRDAFDIWGQGTTVTVSR

SEQ ID NO: 38 - protein, 213 aa, human
SYVLTQPPSVSVAPGETATITCGGDNVGGKSLHWYQVKPGQAPVLVVFDDRDRPSGIPDRFSGANSRDTAALTISRVEAGDEADYYCQVWDDISRLVIFGGGTRLTVLRQPKAAPSVTLFPPSSEELQANKATLVCLISDFYPGAVTVAWKADSSPVKAGVETTTPSRQSNNKYAASSYLSLTPEQWKSHRSYSCQVTHEGSTVEKTVAPTEC

SEQ ID NO: 39 - protein, 120 aa, human
EVQLVESGGGLVQPGGSLRLSCAASGFTFDDYAMYWVRQAPGKGLEWVSGINWNSAIIGYADSVKGRFTISRDNSKNTLYLQMNSLRVEDTAVYFCAKEALYYSAFFDSWGQGTLVTVSR

SEQ ID NO: 40 - protein, 215 aa, human
QSVLTQPPSVSAAPGQKVTISCSGSSSNIGNNYVSWYQQLPGTAPKLLIYDNNKRPSGIPDRFSGSRSGTSATLGITGLQTGDEADYYCGTWDSSLSAWVVGGGTKLTVLGQPKAAPSVTLFPPSSEELRANKATLVCLISDFYPGAVTVAWKADSSPVKAGVETTTPSKQSNNKYAASSYLSLTPEQWKSHRSYSCQVTHEGSTVEKTVAPTEC

SEQ ID NO: 41 - protein, 120 aa, human
EVQLVESGGGLVQPGRSLRLSCAASGFTFGDYAMHWVRQSPGKGLEWVSGINWNGGSTDYADSVEGRFTISRDNAANSLFLQMNSLRAEDTAIYYCARDYADLGSGSDYWGQGTLVTVSS

SEQ ID NO: 42 - protein, 215 aa, human
QSVLTQPPSASGTPGQRVTISCSGSRSNIGSNYVHWYQQLPGAAPKLLIYRNDQRPSGVPDRFSGSRSDTSAFLAISGLRSEDEADYYCASWDDKMSGRLFGGGTKVTVLSQPKAAPSVTLFPPSSEELRANKATLVCLISDFYPGAVTVAWKADSSPVKAGVETTTPSKQSNNKYAASSYLSLTPEQWKSHRSYSCQVTHEGSTVEKTVAPTEC